European Patent Specification EP 3 319 989 B1, published January 8, 2025. Title: Utilisation de fragments Fc mutés en immunothérapie. Applicant: Laboratoire Français du Fractionnement et des Biotechnologies. The sequence listing filed with the application follows.

SEQUENCE LISTING (21 sequences)

SEQ ID NO: 1 - protein, 222 aa, Artificial Sequence
  Fc de l'IgG1 G1m1,17
CPPCPAPELLGGPSVFLFPPKPKDTLMISRTPEVTCVVVDVSHEDPEVKFNWYVDGVEVHNAKTKPREEQYNSTYRVVSVLTVLHQDWLNGKEYKCKVSNKALPAPIEKTISKAKGQPREPQVYTLPPSRDELTKNQVSLTCLVKGFYPSDIAVEWESNGQPENNYKTTPPVLDSDGSFFLYSKLTVDKSRWQQGNVFSCSVMHEALHNHYTQKSLSLSPGK

SEQ ID NO: 2 - protein, 221 aa, Artificial Sequence
  Fc d' IgG2
CPPCPAPPVAGPSVFLFPPKPKDTLMISRTPEVTCVVVDVSHEDPEVQFNWYVDGVEVHNAKTKPREEQFNSTFRVVSVLTVVHQDWLNGKEYKCKVSNKGLPAPIEKTISKTKGQPREPQVYTLPPSREEMTKNQVSLTCLVKGFYPSDIAVEWESNGQPENNYKTTPPMLDSDGSFFLYSKLTVDKSRWQQGNVFSCSVMHEALHNHYTQKSLSLSPGK

SEQ ID NO: 3 - protein, 222 aa, Artificial Sequence
  Fc d' IgG3
CPRCPAPELLGGPSVFLFPPKPKDTLMISRTPEVTCVVVDVSHEDPEVQFKWYVDGVEVHNAKTKPREEQYNSTFRVVSVLTVLHQDWLNGKEYKCKVSNKALPAPIEKTISKTKGQPREPQVYTLPPSREEMTKNQVSLTCLVKGFYPSDIAVEWESSGQPENNYNTTPPMLDSDGSFFLYSKLTVDKSRWQQGNIFSCSVMHEALHNRFTQKSLSLSPGK

SEQ ID NO: 4 - protein, 222 aa, Artificial Sequence
  Fc d' IgG4
CPSCPAPEFLGGPSVFLFPPKPKDTLMISRTPEVTCVVVDVSQEDPEVQFNWYVDGVEVHNAKTKPREEQFNSTYRVVSVLTVLHQDWLNGKEYKCKVSNKGLPSSIEKTISKAKGQPREPQVYTLPPSQEEMTKNQVSLTCLVKGFYPSDIAVEWESNGQPENNYKTTPPVLDSDGSFFLYSRLTVDKSRWQEGNVFSCSVMHEALHNHYTQKSLSLSLGK

SEQ ID NO: 5 - protein, 222 aa, Artificial Sequence
  Fc de l'IgG1 G1m3
CPPCPAPELLGGPSVFLFPPKPKDTLMISRTPEVTCVVVDVSHEDPEVKFNWYVDGVEVHNAKTKPREEQYNSTYRVVSVLTVLHQDWLNGKEYKCKVSNKALPAPIEKTISKAKGQPREPQVYTLPPSREEMTKNQVSLTCLVKGFYPSDIAVEWESNGQPENNYKTTPPVLDSDGSFFLYSKLTVDKSRWQQGNVFSCSVMHEALHNHYTQKSLSLSPGK

SEQ ID NO: 6 - protein, 232 aa, Artificial Sequence
  Fc de l'IgG1 G1m1,17
EPKSCDKTHTCPPCPAPELLGGPSVFLFPPKPKDTLMISRTPEVTCVVVDVSHEDPEVKFNWYVDGVEVHNAKTKPREEQYNSTYRVVSVLTVLHQDWLNGKEYKCKVSNKALPAPIEKTISKAKGQPREPQVYTLPPSRDELTKNQVSLTCLVKGFYPSDIAVEWESNGQPENNYKTTPPVLDSDGSFFLYSKLTVDKSRWQQGNVFSCSVMHEALHNHYTQKSLSLSPGK

SEQ ID NO: 7 - protein, 228 aa, Artificial Sequence
  Fc d' IgG2
ERKCCVECPPCPAPPVAGPSVFLFPPKPKDTLMISRTPEVTCVVVDVSHEDPEVQFNWYVDGVEVHNAKTKPREEQFNSTFRVVSVLTVVHQDWLNGKEYKCKVSNKGLPAPIEKTISKTKGQPREPQVYTLPPSREEMTKNQVSLTCLVKGFYPSDIAVEWESNGQPENNYKTTPPMLDSDGSFFLYSKLTVDKSRWQQGNVFSCSVMHEALHNHYTQKSLSLSPGK

SEQ ID NO: 8 - protein, 279 aa, Artificial Sequence
  Fc d' IgG3
ELKTPLGDTTHTCPRCPEPKSCDTPPPCPRCPEPKSCDTPPPCPRCPEPKSCDTPPPCPRCPAPELLGGPSVFLFPPKPKDTLMISRTPEVTCVVVDVSHEDPEVQFKWYVDGVEVHNAKTKPREEQYNSTFRVVSVLTVLHQDWLNGKEYKCKVSNKALPAPIEKTISKTKGQPREPQVYTLPPSREEMTKNQVSLTCLVKGFYPSDIAVEWESSGQPENNYNTTPPMLDSDGSFFLYSKLTVDKSRWQQGNIFSCSVMHEALHNRFTQKSLSLSPGK

SEQ ID NO: 9 - protein, 229 aa, Artificial Sequence
  Fc d' IgG4
ESKYGPPCPSCPAPEFLGGPSVFLFPPKPKDTLMISRTPEVTCVVVDVSQEDPEVQFNWYVDGVEVHNAKTKPREEQFNSTYRVVSVLTVLHQDWLNGKEYKCKVSNKGLPSSIEKTISKAKGQPREPQVYTLPPSQEEMTKNQVSLTCLVKGFYPSDIAVEWESNGQPENNYKTTPPVLDSDGSFFLYSRLTVDKSRWQEGNVFSCSVMHEALHNHYTQKSLSLSLGK

SEQ ID NO: 10 - protein, 232 aa, Artificial Sequence
  Fc de l'IgG1 G1m3
EPKSCDKTHTCPPCPAPELLGGPSVFLFPPKPKDTLMISRTPEVTCVVVDVSHEDPEVKFNWYVDGVEVHNAKTKPREEQYNSTYRVVSVLTVLHQDWLNGKEYKCKVSNKALPAPIEKTISKAKGQPREPQVYTLPPSREEMTKNQVSLTCLVKGFYPSDIAVEWESNGQPENNYKTTPPVLDSDGSFFLYSKLTVDKSRWQQGNVFSCSVMHEALHNHYTQKSLSLSPGK

SEQ ID NO: 11 - protein, 227 aa, Artificial Sequence
  Fragment Fc muté T5A-74
DKTHTCPPCPAPELLGGPSVFLFPPKPKDTLMISRTPEVTCVVVDVSHEDPEVKFNWYVDGVEVHNAKTKPREEQYNSTYRVVSVLTVLHQDWLDGKEYKCKVSNKALPVPIEKTISKAKGQPREPQVYTLPPSRDELTKDQVSLTCLVKGFYPSDIVVEWESNGQPENNYKTTPPVLDSDGSFFLYSKLTVDKSRWQQGNVFSCSVMHEALHYHYTQKSLSLSPGK

SEQ ID NO: 12 - protein, 227 aa, Artificial Sequence
  Fragment Fc muté T5A-74I
DKTHTCPPCPAPELLGGPSVFLFPPKPKDTLMISRTPEVACVVVDVSHEDPEVKFNWYVDGVEVHNAKTKPREEQYNSTYRVVSVLTVLHQDWLDGKEYKCKVSNKALPVPIEKTISKAKGQPREPQVYTLPPSRDELTKDQVSLTCLVKGFYPSDIVVEWESNGQPENNYKTTPPVLDSDGSFFLYSKLTVDKSRWQQGNVFSCSVMHEALHYHYTQKSLSLSPGK

SEQ ID NO: 13 - protein, 227 aa, Artificial Sequence
  Fragment Fc muté T5A-74J
DKTHTCPPCPAPELLGGPSVFLFPPKPKDTLMISRTPIVTCVVVDVSHEDPEVKFNWYVDGVEVHNAKTKPREEQYNSTYRVVSVLTVLHQDWLDGKEYKCKVSNKALPVPIEKTISKAKGQPREPQVYTLPPSRDELTKDQVSLTCLVKGFYPSDIVVEWESNGQPENNYKTTPPVLDSDGSFFLYSKLTVDKSRWQQGNVFSCSVMHEALHYHYTQKSLSLSPGK

SEQ ID NO: 14 - protein, 227 aa, Artificial Sequence
  Fragment Fc muté T5A-74K
DKTHTCPPCPAPELLGGPSVFLFPPKPKDTLMISRTPEVTCVVVDVSHEDPEVKFNWYVDGVEVHNAKTYPREEQYNSTYRVVSVLTVLHQDWLDGKEYKCKVSNKALPVPIEKTISKAKGQPREPQVYTLPPSRDELTKDQVSLTCLVKGFYPSDIVVEWESNGQPENNYKTTPPVLDSDGSFFLYSKLTVDKSRWQQGNVFSCSVMHEALHYHYTQKSLSLSPGK

SEQ ID NO: 15 - protein, 227 aa, Artificial Sequence
  Fragment Fc muté T5A-74L
DKTHTCPPCPAPELLGGPSVFLFPPKPKDTLMISRTPEVTCVVVDVSHEDPEVKFNWYVDGVEVHNAKTKPREAQYNSTYRVVSVLTVLHQDWLDGKEYKCKVSNKALPVPIEKTISKAKGQPREPQVYTLPPSRDELTKDQVSLTCLVKGFYPSDIVVEWESNGQPENNYKTTPPVLDSDGSFFLYSKLTVDKSRWQQGNVFSCSVMHEALHYHYTQKSLSLSPGK

SEQ ID NO: 16 - protein, 227 aa, Artificial Sequence
  Fragment Fc muté T5A-74M
DKTHTCPPCPAPELLGGPSVFLFPPKPKDTLMISRTPEVTCVVVDVSHEDPEVKFNWYVDGVEVHNAKTKPREEQWNSTYRVVSVLTVLHQDWLDGKEYKCKVSNKALPVPIEKTISKAKGQPREPQVYTLPPSRDELTKDQVSLTCLVKGFYPSDIVVEWESNGQPENNYKTTPPVLDSDGSFFLYSKLTVDKSRWQQGNVFSCSVMHEALHYHYTQKSLSLSPGK

SEQ ID NO: 17 - protein, 227 aa, Artificial Sequence
  Fragment Fc muté ZAC2-85
DKTHTCPPCPAPELLGGPSVFLFPPKPKDTLMISRTPEVACVVVDVSHEDPEVKFNWYVDGVEVHNAKTKPREEQYNSTYRVVSVLTVLHQDWLNGKEYKCKVSNKALPAPIEKTISKAKGQPREPQVYTLPPSRDELTKNQVSLTCLVKGFYPSDIAVEWESNGQPENNYKTTPPVLDSDGSFFLYSKLTVDKSRWQQGNVFSCSVMHEALHNHYTQKSLSLSPGK

SEQ ID NO: 18 - protein, 227 aa, Artificial Sequence
  Fragment Fc muté ZAC3-172
DKTHTCPPCPAPELLGGPSVFLFPPKPKDTLMISRTPEVTCVVVDVSHEDPEVKFNWYVDGVEVHNAKTYPREEQYNSTYRVVSVLTVLHQDWLNGKEYKCKVSNKALPAPIEKTISKAKGQPREPQVYTLPPSRDELTKNQVSLTCLVKGFYPSDIAVEWESNGQPENNYKTTPPVLDSDGSFFLYSKLTVDKSRWQQGNVFSCSVMHEALHNHYTQKSLSLSPGK

SEQ ID NO: 19 - protein, 227 aa, Artificial Sequence
  Fragment Fc muté A3A-184A
DKTHTCPPCPAPELLGGPSVFLFPPKPKDTLMISRTPEVTCVVVDVSHEDPEVKFNWYVDGVEVHNAKTKPREEQYNSTYRVVSVLTVLHQDWLNGKEYKCKVSNKALPAPIENTISKAKGQPREPQVYTLSPSRDELTKNQVSLTCLVKGFYPSDIVVEWESNGQPENNYKTTPPMLDSDGSFFLYSKLTVDKSRWQQGNVFSCSVMHEALHNHYTQKSLSLSPGK

SEQ ID NO: 20 - protein, 227 aa, Artificial Sequence
  Fragment Fc muté A3A-105D
DKTHTCPPCPAPELLGGPSVFLFPPKPKDTLMISRTPEVTCVVVDVSHEDPEVKFNWYVDGVEVHNAKTKPREEQYNSTYRVVSVLTVLHQDWLNDKEYKCKVSNEALPAPIEKTISKAKGQPREPQVYTLPPSRDELTKNQVSLTCLVKGFYPSDIVVEWESNGQPENNYKTTPPVLDSDGSFFLYSKLTVDKSRWQQGNVFSCSVMHEALHNHYTQKSLSLSPGK

SEQ ID NO: 21 - protein, 227 aa, Artificial Sequence
  Fragment Fc muté J3B-118A
DKTHTCPPCPAPELLGGPSVFLFPPKPKDTLMISRTPEVTCVVVDVSHEDPEVKFNWYVDGVEVHNAKTKPREEQYNSTYRVVSVLTVLHQDWLNGKEYKCKVSNKALPAPIEKTISKAKGQPREPQVYTLPPSRDELTKNQVSLTCLVKGFYPSDIVVEWESNGQPENNYKTTPLVLDSDGSFFLYSKLTVDKSRWQQGTVFSCSVMHEALHNHYTQKSLSLSPGK